European Patent Specification EP 3 096 775 B1, published January 11, 2023. Title: SOCS Mimetics for the Treatment of Diseases. Applicant: University of Florida Research Foundation, Inc. Johnson, Howard M. Larkin, Joseph Ahmed, Chulbul M. Jager, Lindsey. The sequence listing filed with the application follows.

SEQUENCE LISTING (54 sequences)

SEQ ID NO: 1 - protein, 16 aa, Artificial sequence
  SOCS1-KIR peptide
DTHFRTFRSHSDYRRI

SEQ ID NO: 2 - protein, 16 aa, Artificial sequence
  SOCS1-KIR2A peptide
DTHARTARSHSDYRRI

SEQ ID NO: 3 - protein, 38 aa, Artificial sequence
  SOCS1-KIR dimer peptide
DTHFRTFRSHSDYRRIGGGGGGDTHFRTFRSHSDYRRI

SEQ ID NO: 4 - protein, 38 aa, Artificial sequence
  SOCS1-KIR2A dimer peptide
DTHARTARSHSDYRRIGGGGGGDTHARTARSHSDYRRI

SEQ ID NO: 5 - protein, 20 aa, Artificial sequence
  amplification primer specific for SOCS1 (forward)
GACACTCACTTCCGCACCTT

SEQ ID NO: 6 - protein, 21 aa, Artificial sequence
  amplification primer specific for SOCS1 (reverse)
GAAGCAGTTCCGTTGGCGACT

SEQ ID NO: 7 - protein, 20 aa, Artificial sequence
  amplification primer specific for beta-actin (forward)
CCACAGCACTGTAGGGTTTA

SEQ ID NO: 8 - protein, 23 aa, Artificial sequence
  amplification primer specific for beta-actin (reverse)
ATTGTCTTTCTTCTGCCGTTCTC

SEQ ID NO: 9 - DNA, 20 bp, Mus musculus
ccttccttcttgggtatgga

SEQ ID NO: 10 - DNA, 20 bp, Mus musculus
ggaggagcaatgatcttgat

SEQ ID NO: 11 - DNA, 23 bp, Mus musculus
aactattttaactcaagtggcat

SEQ ID NO: 12 - DNA, 18 bp, Mus musculus
aggtgtgattcaatgacg

SEQ ID NO: 13 - DNA, 18 bp, Mus musculus
gggagaactttgagtcca

SEQ ID NO: 14 - DNA, 17 bp, Mus musculus
gaaggtcggggtagaaa

SEQ ID NO: 15 - DNA, 17 bp, Mus musculus
actctccaccgcaatga

SEQ ID NO: 16 - DNA, 17 bp, Mus musculus
ctcttcaggaccaggat

SEQ ID NO: 17 - DNA, 22 bp, Mus musculus
acagccactgcattcccagttt

SEQ ID NO: 18 - DNA, 22 bp, Mus musculus
tctcggaaggacttgcagacat

SEQ ID NO: 19 - DNA, 20 bp, Mus musculus
gacactcacttccgcacctt

SEQ ID NO: 20 - DNA, 20 bp, Mus musculus
gaagcagttccgttggcact

SEQ ID NO: 21 - DNA, 19 bp, Homo sapiens
tgcaccaccaactgcttag

SEQ ID NO: 22 - DNA, 18 bp, Homo sapiens
gaggcagggatgatgttc

SEQ ID NO: 23 - DNA, 19 bp, Homo sapiens
gggagcggatgggtgtagg

SEQ ID NO: 24 - DNA, 21 bp, Homo sapiens
agaggtaggaggtgcgagttc

SEQ ID NO: 25 - DNA, 20 bp, Homo sapiens
tgaccagagcatccaaaaga

SEQ ID NO: 26 - DNA, 20 bp, Homo sapiens
ctcttcgacctcgaaacagc

SEQ ID NO: 27 - protein, 25 aa, Artificial sequence
  SOCS1-KIR peptide
RRRRRRRRRDTHFRTFRSHSDYRRI

SEQ ID NO: 28 - protein, 25 aa, Artificial sequence
  SOCS1-KIR2A peptide
RRRRRRRRRDTHARTARSHSDYRRI

SEQ ID NO: 29 - protein, 47 aa, Artificial sequence
  SOCS1-KIR dimer peptide
RRRRRRRRRDTHFRTFRSHSDYRRIGGGGGGDTHFRTFRSHSDYRRI

SEQ ID NO: 30 - protein, 47 aa, Artificial sequence
  SOCS1-KIR dimer peptide
RRRRRRRRRDTHARTARSHSDYRRIGGGGGGDTHARTARSHSDYRRI

SEQ ID NO: 31 - protein, 15 aa, Artificial sequence
  cell-penetrating peptide PTD
RQIKWFQNRRMKWKK

SEQ ID NO: 32 - protein, 11 aa, Artificial sequence
  cell-penetrating peptide TAT
YGRKKRRQRRR

SEQ ID NO: 33 - protein, 18 aa, Artificial sequence
  cell-penetrating peptide SynB1
RGGRLSYSRRRFSTSTGR

SEQ ID NO: 34 - protein, 10 aa, Artificial sequence
  cell-penetrating peptide SynB3
RRLSYSRRRF

SEQ ID NO: 35 - protein, 12 aa, Artificial sequence
  cell-penetrating peptide PTD-4
PIRRRKKLRRLK

SEQ ID NO: 36 - protein, 12 aa, Artificial sequence
  cell-penetrating peptide PTD-5
RRQRRTSKLMKR

SEQ ID NO: 37 - protein, 15 aa, Artificial sequence
  cell-penetrating peptide FHV Coat-(35-49)
RRRRNRTRRNRRRVR

SEQ ID NO: 38 - protein, 19 aa, Artificial sequence
  cell-penetrating peptide BMV Gag-(7-25)
KMTRAQRRAAARRNRWTAR

SEQ ID NO: 39 - protein, 13 aa, Artificial sequence
  cell-penetrating peptide HTLV-II Rex-(4-16)
TRRQRTRRARRNR

SEQ ID NO: 40 - protein, 13 aa, Artificial sequence
  cell-penetrating peptide D-Tat
GRKKRRQRRRPPQ

SEQ ID NO: 41 - protein, 13 aa, Artificial sequence
  cell-penetrating peptide R9-Tat
GRRRRRRRRRPPQ

SEQ ID NO: 42 - protein, 27 aa, Artificial sequence
  cell-penetrating peptide Transportan
GWTLNSAGYLLGKINLKALAALAKKIL

SEQ ID NO: 43 - protein, 17 aa, Artificial sequence
  cell-penetrating peptide MAP
KLALKLALKLALALKLA

SEQ ID NO: 44 - protein, 27 aa, Artificial sequence
  cell-penetrating peptide SBP
MGLGLHLLVLAAALQGAWSQPKKKRKV

SEQ ID NO: 45 - protein, 27 aa, Artificial sequence
  cell-penetrating peptide FBP
GALFLGWLGAAGSTMGAWSQPKKKRKV

SEQ ID NO: 46 - protein, 27 aa, Artificial sequence
  cell-penetrating peptide MPG
GALFLGFLGAAGSTMGAWSQPKKKRKV

SEQ ID NO: 47 - protein, 27 aa, Artificial sequence
  cell-penetrating peptide MPG(delta-NLS)
GALFLGFLGAAGSTMGAWSQPKSKRKV

SEQ ID NO: 48 - protein, 21 aa, Artificial sequence
  cell-penetrating peptide Pep-1
KETWWETWWTEWSQPKKKRKV

SEQ ID NO: 49 - protein, 21 aa, Artificial sequence
  cell-penetrating peptide Pep-2
KETWFETWFTEWSQPKKKRKV

SEQ ID NO: 50 - protein, 12 aa, Artificial sequence
  Tkip peptide
WLVFFVIFYFFR

SEQ ID NO: 51 - protein, 16 aa, Artificial sequence
  SOCS3-KIR peptide
LRLKTFSSKSEYQLVV

SEQ ID NO: 52 - protein, 38 aa, Artificial sequence
  SOCS3-KIR dimer peptide
LRLKTFSSKSEYQLVVGGGGGGLRLKTFSSKSEYQLVV

SEQ ID NO: 53 - protein, 25 aa, Artificial sequence
  SOCS3-KIR peptide
RRRRRRRRRLRLKTFSSKSEYQLVV

SEQ ID NO: 54 - protein, 47 aa, Artificial sequence
  SOCS3-KIR dimer peptide
RRRRRRRRRLRLKTFSSKSEYQLVVGGGGGGLRLKTFSSKSEYQLVV